European Patent Specification EP 3 885 448 B1, published March 22, 2023. Title: ANALYSIS OF CHROMATIN USING A NICKING ENZYME. Applicant: New England Biolabs, Inc. Application Not yet assigned. The sequence listing filed with the application follows.

SEQUENCE LISTING (4 sequences)

SEQ ID NO: 1 - protein, 399 aa, Legionella pneumophila
MKIYSFDTLANADLIIDAVYEGGSSGNASDDPISKIIKGIGNMGGFRSAGQGIFKKLIVLYTNMEDGDWPDSIDTSKGQFIYYGDNKHPGHDIHDTPRQGNATLKMLFDSTHNEKDARRIVPPIFIFVKYPTASSSRSVQFKGVAVPGYPGLSATDDLIAVWKTTNGQRFQNYRAIFTILNIPMVSRKWINSLFDPFGQDNSLNPFYQWKISGKADVLIAPSTKTIRTQIEQMPRTKLEREILQAVFDYFCEAPIKFEACAAKIFQLYDENVLIDEITRSAVDGGKDAIGRYVLGIKEDPVYAEFFLEAKCYQPGLNGQNINSVGVKEVSRLISRIKNRQFGVLVTTSFIAKQAYGEVREDGHPIVFLSGGDISRILIKKGINSTDAVLAWLNSEFSKS

SEQ ID NO: 2 - protein, 159 aa, Nitrolancea hollandica
MNLENLTTRELLAVSRASLRELKRRGVIRSGNAPAGDYAELLVQRATDGELANASQKSWDIRTTEGDRLQVKARVITDEHANGERQLSTIRSWDFDAAVIVLFDDNFRVWRAARVPAAIMKEAAYYSQHVRGYTVYAKDALLNHSEVEDWTEQLRSVEQ

SEQ ID NO: 3 - protein, 168 aa, Bacillus subtilis
MTVSLKKLDDLELTLLYSSLLKELKQRGIIRTNNVVGELGEYLAINFYNKTKGLPKLQAAPTGTQNIDALSIKGDRYSIKTTTGSVTGVFYGMNDPEIREPDIQKFEYVIIVLFDKEYSLKGIYELSWESFIKHKRWHKRMRAWNLTITKALLSDSEIIFEKESKLLN

SEQ ID NO: 4 - protein, 162 aa, Pseudomonas amygdali
MNMEVQDDVYEILREAKILARRYYHLTGKPLGVTGEVAEYEVCRILGLELEQARTAGFDAIETRDGVDLKVQIKGRYFPNSRMRGGRLGSIDLKQPFDIVMLVLLDGDYNAFQIFEAQRPDVEAILTRPGSKSRNERGAVGISQFKAISILRWEREGVDQPA